European Patent Specification EP 4 143 340 B1, published January 21, 2026. Title: MYH11/NDE1 region as epigenetic marker for the identification of endothelial progenitor cells (EPCs). Applicant: Precision for Medicine GmbH. The sequence listing filed with the application follows.

SEQUENCE LISTING (12 sequences)

SEQ ID NO: 1 - DNA, 1083 bp, Homo sapiens
gcgccattgcactccagagcgagactccgtctcaaaaaaaaaaaaaaaaaaaagcaaaatcccagagcagcagagacctcttcatgctttcttgggaagggccctgtgtgcatccttgagtcttgggtatccactccccagtccctgaacatgtacatgcccgtgaagcctccagaaaaggctctgccaggactgtgcttggctttgcggtggtcagcttccaccccgtgtgctgaaaatgcagtttgtagctagacatcactcaagccacgtgcagcccccggcatttgtcagacatcgcagtgagctcatttccttcgcagacaagcctgtgaaagctgaatcatgggaggactggttgccgcgccgcagttaccgtgaactttgtgatctctgacttgtgacccagaccagccaactagaagccaagtacgttctccaggaatgtgcccagatagtggaactgtcatattcattcagtgcagtgtcttcactggacaagggaggacagcactgctgagtgccctaaccacgtaagagtggcttttggcatgaaaggaagaaaaatccaagctacacacacagcctctgccatctcgtcaagatgcagtgataagggcgcacactgttgggtgtcatgtcacatgtgctgcccagaggcaggaaggacagtgggtcaagagatgaggtctatttgtcatcctgatcttggtttcaatgaaagctttgcacaaagatatccaagcctccagattttgcaagaatctcgtggaaatgtgcaagggtttaaaaattggggtgggcagaggggcgcattgggcagaaaagaaatggatactgagacaacacacagctgcgaagctgaaggcatgatacctggtgcatcactgcgaagtttcctgtggggggggccctctgaaacagagagagaatccccggaggttaccatcagcaaacaagaaggagcccggttaagtatattcttaattgttaaagacatttgcttcgatttaataattaaaggcactcttttttattttgagatagtctctgtcacccaggctggagtgcaggggtgcgatc

SEQ ID NO: 2 - DNA, 474 bp, Homo sapiens
gaagggccctgtgtgcatccttgagtcttgggtatccactccccagtccctgaacatgtacatgcccgtgaagcctccagaaaaggctctgccaggactgtgcttggctttgcggtggtcagcttccaccccgtgtgctgaaaatgcagtttgtagctagacatcactcaagccacgtgcagcccccggcatttgtcagacatcgcagtgagctcatttccttcgcagacaagcctgtgaaagctgaatcatgggaggactggttgccgcgccgcagttaccgtgaactttgtgatctctgacttgtgacccagaccagccaactagaagccaagtacgttctccaggaatgtgcccagatagtggaactgtcatattcattcagtgcagtgtcttcactggacaagggaggacagcactgctgagtgccctaaccacgtaagagtggcttttggcatgaaaggaagaaaaatc

SEQ ID NO: 3 - DNA, 22 bp, Homo sapiens
gaagggttttgtgtgtattttt

SEQ ID NO: 4 - DNA, 22 bp, Homo sapiens
aatttttcttcctttcatacca

SEQ ID NO: 5 - DNA, 23 bp, Homo sapiens
ccccaacatttatcaaacatcac

SEQ ID NO: 6 - DNA, 31 bp, Homo sapiens
gggttataagttagagattataaagtttatg

SEQ ID NO: 7 - DNA, 25 bp, Homo sapiens
aattaccacaccacaattaccataa

SEQ ID NO: 8 - DNA, 24 bp, Homo sapiens
atcacaataaactcatttccttca

SEQ ID NO: 9 - DNA, 25 bp, Homo sapiens
aactaattaccacaccacaattacc

SEQ ID NO: 10 - DNA, 21 bp, Homo sapiens
cccgacatttatcaaacatcg

SEQ ID NO: 11 - DNA, 30 bp, Homo sapiens
ggttataagttagagattataaagtttacg

SEQ ID NO: 12 - DNA, 21 bp, Homo sapiens
ttaccgcgccgcaattaccgt